European Patent Application EP 4 606 899 A1, published August 27, 2025. Title: Episomal vector operating in the Bacteroides spp. Applicant: Korea Research Institute of Bioscience and Biotechnology. Application KR. The sequence listing filed with the application follows.

SEQUENCE LISTING (11 sequences)

SEQ ID NO: 1 - DNA, 3146 bp, synthetic construct
  source 1..3146: mol_type = other DNA
accggtcaccctgttttacacccaagaatgtaaagtcgggtgtttttgttttatttaagataatacaaccactacataataaaagagtagcgatattaaaagaatccgatgagaaaagactaatatttatctatccattcagtttgatttctcaggactttacatcgtcctgaaagtatttgttggtaccgaggacgcgtaaacatttacagttgcatgtggcctattgtttttagccgttaaatattttataactattaaatagcgatacaaattgttcgaaactaatattgtttatatcatatattctcgcatgttttaaagctttattaaattgattttttgtaaacagtttttcgtactctttgttaacccatttcattacaaaagtttcatatttttttctctctttaaatgccatttttgctggctttctttttaatacaattaatgtgctatccactttaggttttggatggaaataatacctaggaatttttgctaatatagaaatatctacctctgccattaacagcaatgctagtgatctgtttgtatctaataacattttagcaaaaccatattccactattaaataacttattgtggctgaactttcaaaaacaatttttcgaattatatttgtgcttatgttgtaaggtatgctgccaaatattttatatggattgtggctaggaaatgtaaatttcagtatatcatcatttactatttgatagttaggataatttaagagcttattacgagttacctcacataatttagaatcaatttctatcgccgttacaaaattacatctctttaccaatccagcagtaaaatgacctttccctgcacctatttcaaagatgttatctttttcatctaaacttatgcaattcattattttttctatgtgatattttgaagtaataaaattttgactatcttttatatttactttgttcattataacctctccttaatttattgcatctcttttcgaatatttatgttttttgagaaaagaacgtactcatggttcatcccgatatgcgtatcggtctgtatatcagcaactttctatgtgtttcaactacaatagtcatctattctcatctttctgagtccaccccctgcaaagcccctctttacgacataaaaattcggtcggaaaaggtatgcaaaagatgtttctctctttaagagaaactcttcgggatgcaaaaatatgaaaataactccaattcaccaaattatatagcgacttttttacaaaatgctaaaatttgttgatttccgtcaagcaattgttgagcaaaaatgtcttttacgataaaatgatacctcaatatcaactgtttagcaaaacgatatttctcttaaagagagaaacacctttttgttcaccaatccccgacttttaatcccgcggccatgattgaaaaaggaagagtatgagtattcaacatttccgtgtcgcccttattcccttttttgcggcattttgccttcctgtttttgctcacccagaaacgctggtgaaagtaaaagatgctgaagatcagttgggtgcacgagtgggttacatcgaactggatctcaacagcggtaagatccttgagagttttcgccccgaagaacgttttccaatgatgagcacttttaaagttctgctatgtggcgcggtattatcccgtattgacgccgggcaagagcaactcggtcgccgcatacactattctcagaatgacttggttgagtactcaccagtcacagaaaagcatcttacggatggcatgacagtaagagaattatgcagtgctgccataaccatgagtgataacactgcggccaacttacttctgacaacgatcggaggaccgaaggagctaaccgcttttttgcacaacatgggggatcatgtaactcgccttgatcgttgggaaccggagctgaatgaagccataccaaacgacgagcgtgacaccacgatgcctgtagcaatggcaacaacgttgcgcaaactattaactggcgaactacttactctagcttcccggcaacaattaatagactggatggaggcggataaagttgcaggaccacttctgcgctcggcccttccggctggctggtttattgctgataaatctggagccggtgagcgtgggtctcgcggtatcattgcagcactggggccagatggtaagccctcccgtatcgtagttatctacacgacggggagtcaggcaactatggatgaacgaaatagacagatcgctgagataggtgcctcactgattaagcattggtaactgtcagaccaagtttactcataacgcgtcaattcgagggggatcaattccgtgataggtgggctgcccttcctggttggcttggtttcatcagccatccgcttgccctcatctgttacgccggcggtagccggccagcctcgcagagcaggattcccgttgagcaccgccaggtgcgaataagggacagtgaagaaggaacacccgctcgcgggtgggcctacttcacctatcctgcccggctgacgccgttggatacaccaaggaaagtctacacgaaccctttggcaaaatcctgtatatcgtgcgaaaaaggatggatataccgaaaaaatcgctataatgaccccgaagcagggttatgcagcggaaaacggaattgatccggccacgatgcgtccggcgtagaggatctgaagatcagcagttcaacctgttgatagtacgtactaagctctcatgtttcacgtactaagctctcatgtttaacgtactaagctctcatgtttaacgaactaaaccctcatggctaacgtactaagctctcatggctaacgtactaagctctcatgtttcacgtactaagctctcatgtttgaacaataaaattaatataaatcagcaacttaaatagcctctaaggttttaagttttataagaaaaaaaagaatatataaggcttttaaagcttttaaggtttaacggttgtggacaacaagccagggatgtaacgcactgagaagcccttagagcctctcaaagcaattttgagtgacacaggaacacttaacggctgacatgggaattcccctccaccgcggtggcggccgc

SEQ ID NO: 2 - DNA, 4154 bp, synthetic construct
  source 1..4154: mol_type = other DNA
atcgatagtctatgatgtacacaattagggtttccgacggggtggataaggtgattgccaaatggaagaaatcaaaccccaatttgttcaagaagtataagaaaatctacaaagaattgttagagcaccctaagactgggcttgggcatcccgaagcgttaaggggcggtggggatattacatggtctcgacacattaccgcccatgaccggataatctatgacatttacgaggaagtggtagaggtctacatcttggaggtagaggggcattacaacgataaatgataaaactgttatggtcgaatattgtgtttactggttagagaacggcgagcctatgcacgaggtgttctcttctcttgccgccgccgagatgtactcatgtgcgataagagggaaagaaaacattgaatgggtggaggtgtccgaagaagaaaccattgatttggacgaactggaagacatgttcccggatgacttctgcggcgtgtaatccccttgggtagaaatggggtagaatttgttaggctgtgggggattttctaacacgccggggctttttgctgggcggttggcgtggatgtattcccatgcggcatgtgtatatatagcaagaagtgtccttgtcggacaattcttgcttttctcgctttgctcaaaaagattttaagattacctttgtggcatggaactaagacggaacgaaaagattacattccggtgtaccgaacttgaaaaggacgcacttgcggagcaggcagcccggtgcagtctaagcgtatcggaatactgccggagtttgtcccttggggggcgcccaagggagaggtacaccgaggaggaacggcagcttctccgggacatagcccagttgaaaggaacgctccaacggctgaacaactacttcggtggtcgccagtaccgggaagtgttcgaggagaaccgggcactaattacagagctcaaaaaaatactctcacgatgatagggaaagggaaaagcatatcacatggtgtggcggcattggagtacgacctcgccaaagagataaacgggcaggcagtagccaccgagatagcccggcatgaactttatgggtgtactggtgcggaaatggtgcaggaaatgaaaccgtatcacattgattttccgaacgtaaaaaacaactgcctacgtttcgaggtcagcccctcgatagaggaaagcgccacctttacggatgcggactgggcggaacttggtaacgacttcatgcagcgcatggggttggcgaaccaccagtacatcatcatccggcacagcggtacggagagcaagaaagagcaagcccacctgcacatactggcaaaccgggtttccctttccggggaactgtaccgggacaactggatagggaaaaaggcaacggaagccgccaatgccatagccaaggaacggaactttgtacagtcgcaggacattggcaaagtcaacaaagcggaaatcaaggaagccatggacggcgtattgaagaagatgcagggctttgactttaccaaattcaaggaagaacttggtaagagaggttttaaagtccgggaagccagggcaagcaccgggaaacttaacggctactatgtcacagcccgaagcggtacggagtataaggcaagcgagatagggaaaggctacactctcgcccatatcgagcggacacaaagcaaactgaagtgcaactcaatgaacatatctcatggaaacaaactcacacccggaagcggcagcttccaacgttaagcagggacagtacagcccccggaaaagaaaagatacaacgccaagggtaaacccgcagcttgcggtagaactggtgtatcaagaactaaagcgtgttgaagtctatacgaagcgcatagaggacgcaacagcccgaaaggtacaaatagacgggaaaagccttgaaagtgccgaaaatcgcctaaaaaacgtgttggcggactttgaacggcaggggtacagaatgaaaaacggcggttatgtggacaaacgaatttcgttctactcaatcctttgtgctgttatctccctattgttcgcttgtttcatgtgctatctttggacggatgcagccaaagaccgggacaactacaagcagtattatgaatactaccaagagcaggcaagggaacaaaaggggaataaataaacatctaactttacgaattatgggaacaacggaacacgaagaaccccggttcttcttcatactgaacaagggtgcgaagtccggcggcgaaatcacccatgccgtcctaaacggtagtatcgtttcgaagccggcaggctgggacgcctttcatgggcttgcactggcgagagagaaactaagcagcgaggaaatacaacagcagatgaaagaacttggtgtagaaatggaaatcgttcctctgatttgacaagattacccggagtgtttcagccgggtaatcttgttacttatccttgattttccctttaagggcgtttataatccaccctttcggattgttcttttctcgtgattttccgtttaggagagccagttctccgataaggtcggttatcttttcttgtgccgttatgaatgtctctttgttccggtttatctcttccgatgtgaagccgcaggaataacggaggtactcgtacacatggctgtctatctgatatcgtgctgtaacctttgcttgcaattctttcccttccagttcttcatctctgaactgtggttgatagaccgggtagaacctaaacccggtcaccttgctacgtttgttgtttgggttttcacgcactttcacgtagttgaaagtgtatgggcagctctcatcaagcgcagcctttgctggtttcaaaactctttcctcaaaatgatctattctgtcttttccgttcttgtccttgtatttgtccgcaggtatgccaagacggtctttcaagttttcaagggatatatccaaagggtacacctgcccactcattaacatgtaaaacctaagggaatacccagtaggtagcgcaagagccttgtttaactcaaattctctgtaccccttggcgaacttggtaaacacatcccaaaggtcgttagacacacgaaaggttataatgccagtgcgttttttatattttgggttagatataaatccgcacttccaccattcctcgtcatcttcgtaagtaaaaaaacgtcctgccaaagaatcgagtgcggctatgatttcattgtaatcacgtccggaaaaaataacgtcagatacatgcatttgtgcatcaacatcccaaagtccatgctcaaacttgcgtttcgtgcctgcataatctttcagttttactccctttagttcagcttggcacgcttccagtatgcgaagaactattctttgttcgtgtatggacatgtcttgctgttttgaccatgtatatacccatgaaacaacaacatctttattcttggtaataggtagtttctttttcataaacgattgatttgctgcaaatatacacaatccccacattaaaacaaaaaaagaggggtaaaactcccaaagtgtggggactaatttacttttaaactcccaaagtgtggggactaaactcccaaagtgtggggaaacacatgttctaatccctttatttatgggcgtttgcgaagaagtgatagagcatattacagacgatgcttataacagacaaggggaatttatagagctaagtggttgatttactgtcggaaaaagaaaaacgatagggaaaaagagcaaagcaaaaccaaccaacgggcggtaggattggaaacgggtttttatggcgtgtacacgtttgtgtacaaaatgtttgtattttattgaaatatagctatctttgtgctgaatttaaaagcaaacagatatggaagcattatcagtaagagaataccgtaacaacctcgcagcgtctttcaccaaagctgacaatggcgagcaggtactaattcgcaggaaaaacgagatttacgctttggtaaaagttggtcgtgaagatttgatgataaccccggagctgcaagcaaggattgacaaggcaagggaagaaatcaaatccggaaagtgtgttaccctcaaaagcagtgaggatattgacgcttatttcgat

SEQ ID NO: 3 - DNA, 7300 bp, synthetic construct
  source 1..7300: mol_type = other DNA
atcgatagtctatgatgtacacaattagggtttccgacggggtggataaggtgattgccaaatggaagaaatcaaaccccaatttgttcaagaagtataagaaaatctacaaagaattgttagagcaccctaagactgggcttgggcatcccgaagcgttaaggggcggtggggatattacatggtctcgacacattaccgcccatgaccggataatctatgacatttacgaggaagtggtagaggtctacatcttggaggtagaggggcattacaacgataaatgataaaactgttatggtcgaatattgtgtttactggttagagaacggcgagcctatgcacgaggtgttctcttctcttgccgccgccgagatgtactcatgtgcgataagagggaaagaaaacattgaatgggtggaggtgtccgaagaagaaaccattgatttggacgaactggaagacatgttcccggatgacttctgcggcgtgtaatccccttgggtagaaatggggtagaatttgttaggctgtgggggattttctaacacgccggggctttttgctgggcggttggcgtggatgtattcccatgcggcatgtgtatatatagcaagaagtgtccttgtcggacaattcttgcttttctcgctttgctcaaaaagattttaagattacctttgtggcatggaactaagacggaacgaaaagattacattccggtgtaccgaacttgaaaaggacgcacttgcggagcaggcagcccggtgcagtctaagcgtatcggaatactgccggagtttgtcccttggggggcgcccaagggagaggtacaccgaggaggaacggcagcttctccgggacatagcccagttgaaaggaacgctccaacggctgaacaactacttcggtggtcgccagtaccgggaagtgttcgaggagaaccgggcactaattacagagctcaaaaaaatactctcacgatgatagggaaagggaaaagcatatcacatggtgtggcggcattggagtacgacctcgccaaagagataaacgggcaggcagtagccaccgagatagcccggcatgaactttatgggtgtactggtgcggaaatggtgcaggaaatgaaaccgtatcacattgattttccgaacgtaaaaaacaactgcctacgtttcgaggtcagcccctcgatagaggaaagcgccacctttacggatgcggactgggcggaacttggtaacgacttcatgcagcgcatggggttggcgaaccaccagtacatcatcatccggcacagcggtacggagagcaagaaagagcaagcccacctgcacatactggcaaaccgggtttccctttccggggaactgtaccgggacaactggatagggaaaaaggcaacggaagccgccaatgccatagccaaggaacggaactttgtacagtcgcaggacattggcaaagtcaacaaagcggaaatcaaggaagccatggacggcgtattgaagaagatgcagggctttgactttaccaaattcaaggaagaacttggtaagagaggttttaaagtccgggaagccagggcaagcaccgggaaacttaacggctactatgtcacagcccgaagcggtacggagtataaggcaagcgagatagggaaaggctacactctcgcccatatcgagcggacacaaagcaaactgaagtgcaactcaatgaacatatctcatggaaacaaactcacacccggaagcggcagcttccaacgttaagcagggacagtacagcccccggaaaagaaaagatacaacgccaagggtaaacccgcagcttgcggtagaactggtgtatcaagaactaaagcgtgttgaagtctatacgaagcgcatagaggacgcaacagcccgaaaggtacaaatagacgggaaaagccttgaaagtgccgaaaatcgcctaaaaaacgtgttggcggactttgaacggcaggggtacagaatgaaaaacggcggttatgtggacaaacgaatttcgttctactcaatcctttgtgctgttatctccctattgttcgcttgtttcatgtgctatctttggacggatgcagccaaagaccgggacaactacaagcagtattatgaatactaccaagagcaggcaagggaacaaaaggggaataaataaacatctaactttacgaattatgggaacaacggaacacgaagaaccccggttcttcttcatactgaacaagggtgcgaagtccggcggcgaaatcacccatgccgtcctaaacggtagtatcgtttcgaagccggcaggctgggacgcctttcatgggcttgcactggcgagagagaaactaagcagcgaggaaatacaacagcagatgaaagaacttggtgtagaaatggaaatcgttcctctgatttgacaagattacccggagtgtttcagccgggtaatcttgttacttatccttgattttccctttaagggcgtttataatccaccctttcggattgttcttttctcgtgattttccgtttaggagagccagttctccgataaggtcggttatcttttcttgtgccgttatgaatgtctctttgttccggtttatctcttccgatgtgaagccgcaggaataacggaggtactcgtacacatggctgtctatctgatatcgtgctgtaacctttgcttgcaattctttcccttccagttcttcatctctgaactgtggttgatagaccgggtagaacctaaacccggtcaccttgctacgtttgttgtttgggttttcacgcactttcacgtagttgaaagtgtatgggcagctctcatcaagcgcagcctttgctggtttcaaaactctttcctcaaaatgatctattctgtcttttccgttcttgtccttgtatttgtccgcaggtatgccaagacggtctttcaagttttcaagggatatatccaaagggtacacctgcccactcattaacatgtaaaacctaagggaatacccagtaggtagcgcaagagccttgtttaactcaaattctctgtaccccttggcgaacttggtaaacacatcccaaaggtcgttagacacacgaaaggttataatgccagtgcgttttttatattttgggttagatataaatccgcacttccaccattcctcgtcatcttcgtaagtaaaaaaacgtcctgccaaagaatcgagtgcggctatgatttcattgtaatcacgtccggaaaaaataacgtcagatacatgcatttgtgcatcaacatcccaaagtccatgctcaaacttgcgtttcgtgcctgcataatctttcagttttactccctttagttcagcttggcacgcttccagtatgcgaagaactattctttgttcgtgtatggacatgtcttgctgttttgaccatgtatatacccatgaaacaacaacatctttattcttggtaataggtagtttctttttcataaacgattgatttgctgcaaatatacacaatccccacattaaaacaaaaaaagaggggtaaaactcccaaagtgtggggactaatttacttttaaactcccaaagtgtggggactaaactcccaaagtgtggggaaacacatgttctaatccctttatttatgggcgtttgcgaagaagtgatagagcatattacagacgatgcttataacagacaaggggaatttatagagctaagtggttgatttactgtcggaaaaagaaaaacgatagggaaaaagagcaaagcaaaaccaaccaacgggcggtaggattggaaacgggtttttatggcgtgtacacgtttgtgtacaaaatgtttgtattttattgaaatatagctatctttgtgctgaatttaaaagcaaacagatatggaagcattatcagtaagagaataccgtaacaacctcgcagcgtctttcaccaaagctgacaatggcgagcaggtactaattcgcaggaaaaacgagatttacgctttggtaaaagttggtcgtgaagatttgatgataaccccggagctgcaagcaaggattgacaaggcaagggaagaaatcaaatccggaaagtgtgttaccctcaaaagcagtgaggatattgacgcttatttcgataccggtcaccctgttttacacccaagaatgtaaagtcgggtgtttttgttttatttaagataatacaaccactacataataaaagagtagcgatattaaaagaatccgatgagaaaagactaatatttatctatccattcagtttgatttctcaggactttacatcgtcctgaaagtatttgttggtaccgaggacgcgtaaacatttacagttgcatgtggcctattgtttttagccgttaaatattttataactattaaatagcgatacaaattgttcgaaactaatattgtttatatcatatattctcgcatgttttaaagctttattaaattgattttttgtaaacagtttttcgtactctttgttaacccatttcattacaaaagtttcatatttttttctctctttaaatgccatttttgctggctttctttttaatacaattaatgtgctatccactttaggttttggatggaaataatacctaggaatttttgctaatatagaaatatctacctctgccattaacagcaatgctagtgatctgtttgtatctaataacattttagcaaaaccatattccactattaaataacttattgtggctgaactttcaaaaacaatttttcgaattatatttgtgcttatgttgtaaggtatgctgccaaatattttatatggattgtggctaggaaatgtaaatttcagtatatcatcatttactatttgatagttaggataatttaagagcttattacgagttacctcacataatttagaatcaatttctatcgccgttacaaaattacatctctttaccaatccagcagtaaaatgacctttccctgcacctatttcaaagatgttatctttttcatctaaacttatgcaattcattattttttctatgtgatattttgaagtaataaaattttgactatcttttatatttactttgttcattataacctctccttaatttattgcatctcttttcgaatatttatgttttttgagaaaagaacgtactcatggttcatcccgatatgcgtatcggtctgtatatcagcaactttctatgtgtttcaactacaatagtcatctattctcatctttctgagtccaccccctgcaaagcccctctttacgacataaaaattcggtcggaaaaggtatgcaaaagatgtttctctctttaagagaaactcttcgggatgcaaaaatatgaaaataactccaattcaccaaattatatagcgacttttttacaaaatgctaaaatttgttgatttccgtcaagcaattgttgagcaaaaatgtcttttacgataaaatgatacctcaatatcaactgtttagcaaaacgatatttctcttaaagagagaaacacctttttgttcaccaatccccgacttttaatcccgcggccatgattgaaaaaggaagagtatgagtattcaacatttccgtgtcgcccttattcccttttttgcggcattttgccttcctgtttttgctcacccagaaacgctggtgaaagtaaaagatgctgaagatcagttgggtgcacgagtgggttacatcgaactggatctcaacagcggtaagatccttgagagttttcgccccgaagaacgttttccaatgatgagcacttttaaagttctgctatgtggcgcggtattatcccgtattgacgccgggcaagagcaactcggtcgccgcatacactattctcagaatgacttggttgagtactcaccagtcacagaaaagcatcttacggatggcatgacagtaagagaattatgcagtgctgccataaccatgagtgataacactgcggccaacttacttctgacaacgatcggaggaccgaaggagctaaccgcttttttgcacaacatgggggatcatgtaactcgccttgatcgttgggaaccggagctgaatgaagccataccaaacgacgagcgtgacaccacgatgcctgtagcaatggcaacaacgttgcgcaaactattaactggcgaactacttactctagcttcccggcaacaattaatagactggatggaggcggataaagttgcaggaccacttctgcgctcggcccttccggctggctggtttattgctgataaatctggagccggtgagcgtgggtctcgcggtatcattgcagcactggggccagatggtaagccctcccgtatcgtagttatctacacgacggggagtcaggcaactatggatgaacgaaatagacagatcgctgagataggtgcctcactgattaagcattggtaactgtcagaccaagtttactcataacgcgtcaattcgagggggatcaattccgtgataggtgggctgcccttcctggttggcttggtttcatcagccatccgcttgccctcatctgttacgccggcggtagccggccagcctcgcagagcaggattcccgttgagcaccgccaggtgcgaataagggacagtgaagaaggaacacccgctcgcgggtgggcctacttcacctatcctgcccggctgacgccgttggatacaccaaggaaagtctacacgaaccctttggcaaaatcctgtatatcgtgcgaaaaaggatggatataccgaaaaaatcgctataatgaccccgaagcagggttatgcagcggaaaacggaattgatccggccacgatgcgtccggcgtagaggatctgaagatcagcagttcaacctgttgatagtacgtactaagctctcatgtttcacgtactaagctctcatgtttaacgtactaagctctcatgtttaacgaactaaaccctcatggctaacgtactaagctctcatggctaacgtactaagctctcatgtttcacgtactaagctctcatgtttgaacaataaaattaatataaatcagcaacttaaatagcctctaaggttttaagttttataagaaaaaaaagaatatataaggcttttaaagcttttaaggtttaacggttgtggacaacaagccagggatgtaacgcactgagaagcccttagagcctctcaaagcaattttgagtgacacaggaacacttaacggctgacatgggaattcccctccaccgcggtggcggccgc

SEQ ID NO: 4 - DNA, 21 bp, synthetic construct
  source 1..21: mol_type = other DNA
catcgttcgtcagcagtaaca

SEQ ID NO: 5 - DNA, 20 bp, synthetic construct
  source 1..20: mol_type = other DNA
ccaagaaaaagggacagtgg

SEQ ID NO: 6 - DNA, 20 bp, synthetic construct
  source 1..20: mol_type = other DNA
ggataaagttgcaggaccac

SEQ ID NO: 7 - DNA, 20 bp, synthetic construct
  source 1..20: mol_type = other DNA
tcagcaataaaccagccagc

SEQ ID NO: 8 - DNA, 642 bp, synthetic construct
  source 1..642: mol_type = other DNA
acgactagcaatcctcgtatgcaagtgcgtgtgagcctggagaagttaagcctgtatatgcgtcagtcgccgaatgtacttacgcaggacgacccgcgccctttaccgaaaccgaaaaaatgggcagactttgagattccctttaaagtagaggcagcaccgactcctaagtccggctacatcgacgccttaaccttcaagttctatatcgcggtagtgaatcctgaccgctctcgtcagtacttgaaattgtacaaagaggtaaagtacgttaacgtgccagttggggaaaacacgtacgccagcgtctatttgagcccatcttctgtcaaacgtattacaggagtggaaggaggtcgcggtaaatgggttaaatatcaaggagtcgtcgtcgagtataatgggaagattgttgcgacatattcctcggaacgtggaaagatggagaaatggtggaccattcagtcaccctcgatcgttgaaacaagctattatccgttattaaacaaggatgaaactcctttcagtgtattttggtacgatcgctacccagagatcatgcgcccaaactcccaacaagcagcatcatctagcgtaccagccccttttggcacaccagtggagccaccagcagacggagag

SEQ ID NO: 9 - DNA, 951 bp, synthetic construct
  source 1..951: mol_type = other DNA
atgtctaactggatcactgacaacaaaccggctgctatggtagctggtgtaggtttgttgttgttcttgggtttgtctgctactggttacatcgtaaactctaaacgttctgaattggacaaaaaaatctctatcgctgctaaagaaatcaaatctgctaacgctgctgaaatcactccgtctcgttcttctaacgaagaattggaaaaagaattgaaccgttacgctaaagctgtaggttctttggaaactgcttacaaaccgttcttggcttcttctgctttggtaccgactactccgactgctttccagaacgaattgaaaactttccgtgactctttgatctcttcttgtaaaaaaaaaaacatcttgatcactgacacttcttcttggttgggtttccaggtatactctactcaggctccgtctgtacaggctgcttctactttgggtttcgaattgaaagctatcaactctttggtaaacaaattggctgaatgtggtttgtctaaattcatcaaagtataccgtccgcagttgccgatcgaaactccggctaacaacccggaagaatctgacgaagctgaccaggctccgtggactccgatgccgttggaaatcgctttccagggtgaccgtgaatctgtattgaaagctatgaacgctatcactggtatgcaggactacttgttcactgtaaactctatccgtatccgtaacgaacgtatgatgccgccgccgatcgctaacccggctgctgctaaaccggctgctgctcagccggctactggtgctgcttctttgactccggctgacgaagctgctgctccggctgctccggctatccagcaggtaatcaaaccgtacatgggtaaagaacaggtattcgtacaggtatctttgaacttggtacacttcaaccagccgaaagctcaggaaccgtctgaagac

SEQ ID NO: 10 - DNA, 795 bp, unidentified
  source 1..795: mol_type = genomic DNA
ttataccgctactattccggcaatatgtggatgcgggtcgtagttcaccagttcgaagtcttcgaactggaagtcatagatactcttcacatccggattaattttcatttgaggcaatgcgcgtggttcgcggctaagctgcaatttgacctgatccaagtggttcagatagatatgggcatcgccaagtgtatggataaattcacccgctttcagtcctgtcacctgcgccatcatttgtagcagcagtgcatatgatgcgatattgaacgggactccgagaaatatatccgcgctgcgctggtaaagttgcaggctcagccgaccgtctgccacgtaaaactggaagaaggcatgacagggaggcaggttcatattctttaaatcggctacattccaggcgctgacaatgatacggcgggagtcgggattgtgcttgatcgtctctaccgcttcgctgatctggtcgatgaatccgccgtcgtagtcgggccacgaacgccactgatagccatagatatgccctaaatcaccgttctcgtccgcccattcgttccagatgcgtacaccgtgttcttgcagatatttcgcgttcgtatcaccttgcagaaaccagagtaactcgtagatgattgatttcagatgcagttttttggtggtcagacacgggaaaccctcgtcgaggttgaaacgcatctgatgtccgaacacactgatcgttccggttcctgtacggtcacttttctcagttccttcagttaatacgcgattgagtaaatctaaatattgtttcat

SEQ ID NO: 11 - DNA, 9218 bp, synthetic construct
  source 1..9218: mol_type = other DNA
atcgatagtctatgatgtacacaattagggtttccgacggggtggataaggtgattgccaaatggaagaaatcaaaccccaatttgttcaagaagtataagaaaatctacaaagaattgttagagcaccctaagactgggcttgggcatcccgaagcgttaaggggcggtggggatattacatggtctcgacacattaccgcccatgaccggataatctatgacatttacgaggaagtggtagaggtctacatcttggaggtagaggggcattacaacgataaatgataaaactgttatggtcgaatattgtgtttactggttagagaacggcgagcctatgcacgaggtgttctcttctcttgccgccgccgagatgtactcatgtgcgataagagggaaagaaaacattgaatgggtggaggtgtccgaagaagaaaccattgatttggacgaactggaagacatgttcccggatgacttctgcggcgtgtaatccccttgggtagaaatggggtagaatttgttaggctgtgggggattttctaacacgccggggctttttgctgggcggttggcgtggatgtattcccatgcggcatgtgtatatatagcaagaagtgtccttgtcggacaattcttgcttttctcgctttgctcaaaaagattttaagattacctttgtggcatggaactaagacggaacgaaaagattacattccggtgtaccgaacttgaaaaggacgcacttgcggagcaggcagcccggtgcagtctaagcgtatcggaatactgccggagtttgtcccttggggggcgcccaagggagaggtacaccgaggaggaacggcagcttctccgggacatagcccagttgaaaggaacgctccaacggctgaacaactacttcggtggtcgccagtaccgggaagtgttcgaggagaaccgggcactaattacagagctcaaaaaaatactctcacgatgatagggaaagggaaaagcatatcacatggtgtggcggcattggagtacgacctcgccaaagagataaacgggcaggcagtagccaccgagatagcccggcatgaactttatgggtgtactggtgcggaaatggtgcaggaaatgaaaccgtatcacattgattttccgaacgtaaaaaacaactgcctacgtttcgaggtcagcccctcgatagaggaaagcgccacctttacggatgcggactgggcggaacttggtaacgacttcatgcagcgcatggggttggcgaaccaccagtacatcatcatccggcacagcggtacggagagcaagaaagagcaagcccacctgcacatactggcaaaccgggtttccctttccggggaactgtaccgggacaactggatagggaaaaaggcaacggaagccgccaatgccatagccaaggaacggaactttgtacagtcgcaggacattggcaaagtcaacaaagcggaaatcaaggaagccatggacggcgtattgaagaagatgcagggctttgactttaccaaattcaaggaagaacttggtaagagaggttttaaagtccgggaagccagggcaagcaccgggaaacttaacggctactatgtcacagcccgaagcggtacggagtataaggcaagcgagatagggaaaggctacactctcgcccatatcgagcggacacaaagcaaactgaagtgcaactcaatgaacatatctcatggaaacaaactcacacccggaagcggcagcttccaacgttaagcagggacagtacagcccccggaaaagaaaagatacaacgccaagggtaaacccgcagcttgcggtagaactggtgtatcaagaactaaagcgtgttgaagtctatacgaagcgcatagaggacgcaacagcccgaaaggtacaaatagacgggaaaagccttgaaagtgccgaaaatcgcctaaaaaacgtgttggcggactttgaacggcaggggtacagaatgaaaaacggcggttatgtggacaaacgaatttcgttctactcaatcctttgtgctgttatctccctattgttcgcttgtttcatgtgctatctttggacggatgcagccaaagaccgggacaactacaagcagtattatgaatactaccaagagcaggcaagggaacaaaaggggaataaataaacatctaactttacgaattatgggaacaacggaacacgaagaaccccggttcttcttcatactgaacaagggtgcgaagtccggcggcgaaatcacccatgccgtcctaaacggtagtatcgtttcgaagccggcaggctgggacgcctttcatgggcttgcactggcgagagagaaactaagcagcgaggaaatacaacagcagatgaaagaacttggtgtagaaatggaaatcgttcctctgatttgacaagattacccggagtgtttcagccgggtaatcttgttacttatccttgattttccctttaagggcgtttataatccaccctttcggattgttcttttctcgtgattttccgtttaggagagccagttctccgataaggtcggttatcttttcttgtgccgttatgaatgtctctttgttccggtttatctcttccgatgtgaagccgcaggaataacggaggtactcgtacacatggctgtctatctgatatcgtgctgtaacctttgcttgcaattctttcccttccagttcttcatctctgaactgtggttgatagaccgggtagaacctaaacccggtcaccttgctacgtttgttgtttgggttttcacgcactttcacgtagttgaaagtgtatgggcagctctcatcaagcgcagcctttgctggtttcaaaactctttcctcaaaatgatctattctgtcttttccgttcttgtccttgtatttgtccgcaggtatgccaagacggtctttcaagttttcaagggatatatccaaagggtacacctgcccactcattaacatgtaaaacctaagggaatacccagtaggtagcgcaagagccttgtttaactcaaattctctgtaccccttggcgaacttggtaaacacatcccaaaggtcgttagacacacgaaaggttataatgccagtgcgttttttatattttgggttagatataaatccgcacttccaccattcctcgtcatcttcgtaagtaaaaaaacgtcctgccaaagaatcgagtgcggctatgatttcattgtaatcacgtccggaaaaaataacgtcagatacatgcatttgtgcatcaacatcccaaagtccatgctcaaacttgcgtttcgtgcctgcataatctttcagttttactccctttagttcagcttggcacgcttccagtatgcgaagaactattctttgttcgtgtatggacatgtcttgctgttttgaccatgtatatacccatgaaacaacaacatctttattcttggtaataggtagtttctttttcataaacgattgatttgctgcaaatatacacaatccccacattaaaacaaaaaaagaggggtaaaactcccaaagtgtggggactaatttacttttaaactcccaaagtgtggggactaaactcccaaagtgtggggaaacacatgttctaatccctttatttatgggcgtttgcgaagaagtgatagagcatattacagacgatgcttataacagacaaggggaatttatagagctaagtggttgatttactgtcggaaaaagaaaaacgatagggaaaaagagcaaagcaaaaccaaccaacgggcggtaggattggaaacgggtttttatggcgtgtacacgtttgtgtacaaaatgtttgtattttattgaaatatagctatctttgtgctgaatttaaaagcaaacagatatggaagcattatcagtaagagaataccgtaacaacctcgcagcgtctttcaccaaagctgacaatggcgagcaggtactaattcgcaggaaaaacgagatttacgctttggtaaaagttggtcgtgaagatttgatgataaccccggagctgcaagcaaggattgacaaggcaagggaagaaatcaaatccggaaagtgtgttaccctcaaaagcagtgaggatattgacgcttatttcgataccggtcaccctgttttacacccaagaatgtaaagtcgggtgtttttgttttatttaagataatacaaccactacataataaaagagtagcgatattaattagccgttaaatattttataactattaaatagcgatacaaattgttcgaaactaatattgtttatatcatatattctcgcatgttttaaagctttattaaattgattttttgtaaacagtttttcgtactctttgttaacccatttcattacaaaagtttcatatttttttctctctttaaatgccatttttgctggctttctttttaatacaattaatgtgctatccactttaggttttggatggaaataatacctaggaatttttgctaatatagaaatatctacctctgccattaacagcaatgctagtgatctgtttgtatctaataacattttagcaaaaccatattccactattaaataacttattgtggctgaactttcaaaaacaatttttcgaattatatttgtgcttatgttgtaaggtatgctgccaaatattttatatggattgtggctaggaaatgtaaatttcagtatatcatcatttactatttgatagttaggataatttaagagcttattacgagttacctcacataatttagaatcaatttctatcgccgttacaaaattacatctctttaccaatccagcagtaaaatgacctttccctgcacctatttcaaagatgttatctttttcatctaaacttatgcaattcattattttttctatgtgatattttgaagtaataaaattttgactatcttttatatttactttgttcataattgggtgcgtttgaaattctacacccaaatatacacccaattattgagatagcaaaagacatttagaaacatttacttttactctatattgtaatttacacttgattatcagtcgtttgcagttttatgatattctgtgaaagtataagttcgagagaagaatccgatgagaaaagactaatatttatctatccattcagtttgatttctcaggactttacatcgtcctgaaagtatttgttggtaccgaggacgcgtaaacatttacagttgcatgtggcctattgtttttataccgctactattccggcaatatgtggatgcgggtcgtagttcaccagttcgaagtcttcgaactggaagtcatagatactcttcacatccggattaattttcatttgaggcaatgcgcgtggttcgcggctaagctgcaatttgacctgatccaagtggttcagatagatatgggcatcgccaagtgtatggataaattcacccgctttcagtcctgtcacctgcgccatcatttgtagcagcagtgcatatgatgcgatattgaacgggactccgagaaatatatccgcgctgcgctggtaaagttgcaggctcagccgaccgtctgccacgtaaaactggaagaaggcatgacagggaggcaggttcatattctttaaatcggctacattccaggcgctgacaatgatacggcgggagtcgggattgtgcttgatcgtctctaccgcttcgctgatctggtcgatgaatccgccgtcgtagtcgggccacgaacgccactgatagccatagatatgccctaaatcaccgttctcgtccgcccattcgttccagatgcgtacaccgtgttcttgcagatatttcgcgttcgtatcaccttgcagaaaccagagtaactcgtagatgattgatttcagatgcagttttttggtggtcagacacgggaaaccctcgtcgaggttgaaacgcatctgatgtccgaacacactgatcgttccggttcctgtacggtcacttttctcagttccttcagttaatacgcgattgagtaaatctaaatattgtttcattataacctctccttaatttattgcatctcttttcgaatatttatgttttttgagaaaagaacgtactcatggttcatcccgatatgcgtatcggtctgtatatcagcaactttctatgtgtttcaactacaatagtcatctattctcatctttctgagtccaccccctgcaaagcccctctttacgacataaaaattcggtcggaaaaggtatgcaaaagatgtttctctctttaagagaaactcttcgggatgcaaaaatatgaaaataactccaattcaccaaattatatagcgacttttttacaaaatgctaaaatttgttgatttccgtcaagcaattgttgagcaaaaatgtcttttacgataaaatgatacctcaatatcaactgtttagcaaaacgatatttctcttaaagagagaaacacctttttgttcaccaatccccgacttttaatcccgcggccatgattgaaaaaggaagagtatgagtattcaacatttccgtgtcgcccttattcccttttttgcggcattttgccttcctgtttttgctcacccagaaacgctggtgaaagtaaaagatgctgaagatcagttgggtgcacgagtgggttacatcgaactggatctcaacagcggtaagatccttgagagttttcgccccgaagaacgttttccaatgatgagcacttttaaagttctgctatgtggcgcggtattatcccgtattgacgccgggcaagagcaactcggtcgccgcatacactattctcagaatgacttggttgagtactcaccagtcacagaaaagcatcttacggatggcatgacagtaagagaattatgcagtgctgccataaccatgagtgataacactgcggccaacttacttctgacaacgatcggaggaccgaaggagctaaccgcttttttgcacaacatgggggatcatgtaactcgccttgatcgttgggaaccggagctgaatgaagccataccaaacgacgagcgtgacaccacgatgcctgtagcaatggcaacaacgttgcgcaaactattaactggcgaactacttactctagcttcccggcaacaattaatagactggatggaggcggataaagttgcaggaccacttctgcgctcggcccttccggctggctggtttattgctgataaatctggagccggtgagcgtgggtctcgcggtatcattgcagcactggggccagatggtaagccctcccgtatcgtagttatctacacgacggggagtcaggcaactatggatgaacgaaatagacagatcgctgagataggtgcctcactgattaagcattggtaactgtcagaccaagtttactcataacgcgtcaattcgagggggatcaattccgtgataggtgggctgcccttcctggttggcttggtttcatcagccatccgcttgccctcatctgttacgccggcggtagccggccagcctcgcagagcaggattcccgttgagcaccgccaggtgcgaataagggacagtgaagaaggaacacccgctcgcgggtgggcctacttcacctatcctgcccggctgacgccgttggatacaccaaggaaagtctacacgaaccctttggcaaaatcctgtatatcgtgcgaaaaaggatggatataccgaaaaaatcgctataatgaccccgaagcagggttatgcagcggaaaacggaattgatccggccacgatgcgtccggcgtagaggatctgaagatcagcagttcaacctgttgatagtacgtactaagctctcatgtttcacgtactaagctctcatgtttaacgtactaagctctcatgtttaacgaactaaaccctcatggctaacgtactaagctctcatggctaacgtactaagctctcatgtttcacgtactaagctctcatgtttgaacaataaaattaatataaatcagcaacttaaatagcctctaaggttttaagttttataagaaaaaaaagaatatataaggcttttaaagcttttaaggtttaacggttgtggacaacaagccagggatgtaacgcactgagaagcccttagagcctctcaaagcaattttgagtgacacaggaacacttaacggctgacatgggaattcccctccaccgcggtggcggccgctgatctggaagaagcaatgaaagctgctgttaagtctccgaatcaggtattgttcctgacaggtgtattcccatccggtaaacgcggatactttgcagttgatctgactcaggaataaattataaattaaggtaagaagattgtaggataagctaatgaaatagaaaaaggatgccgtcacacaacttgtcggcattcttttttgttttattagttgaaaatatagtgaaaaagttgcctaaatatgtatgttaacaaattatttgtcgtaactttgcactccaaatctgtttttaacatatggcactaatggtttttactctggaagattttgttggcgattggcgtcagaccgcgggttataatttggatcaagtcctggaacagggtggcgtaagctctctgttccagaacctgggtgtgagcgtgacgccgattcagcgcatcgttctgtccggcgagaacggtctgaaaattgatattcatgtgatcatcccgtacgaaggcctgagcggtgaccaaatgggtcaaatcgagaaaatctttaaagtcgtctacccagttgacgatcaccacttcaaggttatcttgcattacggtacgctggtgattgatggtgtgaccccgaatatgattgactatttcggccgtccgtatgaaggcattgccgtttttgacggtaaaaagatcaccgtcaccggtaccctgtggaatggcaataagattattgacgagcgtctgattaacccggacggcagcctgctgttccgcgtgaccatcaacggtgtcacgggttggcgtctgtgcgagcgcatcctggcataatgaactgcacttgctttgataattaatgataaacaatctaaaagcactctaatcgttatcggagtgcttttagattactaatcaaattgcttctactaattgcctatcttccagtgatggaacagcatttgtgcattgg